European Patent Specification EP 3 538 136 B1, published June 10, 2026. Title: SUBCUTANEOUS DELIVERY OF MESSENGER RNA. Applicant: Translate Bio, Inc. The sequence listing filed with the application follows.

SEQUENCE LISTING (8 sequences)

SEQ ID NO: 1 - RNA, 140 nt, Artificial Sequence
  chemically synthesized oligonucleotide
ggacagaucgccuggagacgccauccacgcuguuuugaccuccauagaagacaccgggaccgauccagccuccgcggccgggaacggugcauuggaacgcggauuccccgugccaagagugacucaccguccuugacacg

SEQ ID NO: 2 - RNA, 105 nt, Artificial Sequence
  chemically synthesized oligonucleotide
cggguggcaucccugugaccccuccccagugccucuccuggcccuggaaguugccacuccagugcccaccagccuuguccuaauaaaauuaaguugcaucaagcu

SEQ ID NO: 3 - RNA, 105 nt, Artificial Sequence
  chemically synthesized oligonucleotide
ggguggcaucccugugaccccuccccagugccucuccuggcccuggaaguugccacuccagugcccaccagccuuguccuaauaaaauuaaguugcaucaaagcu

SEQ ID NO: 4 - RNA, 1310 nt, Artificial Sequence
  chemically synthesized oligonucleotide
ggacagaucgccuggagacgccauccacgcuguuuugaccuccauagaagacaccgggaccgauccagccuccgcggccgggaacggugcauuggaacgcggauuccccgugccaagagugacucaccguccuugacacgaugcuguucaaccuucggaucuugcugaacaacgcugcguuccggaauggucacaacuucaugguccggaacuucagaugcggccagccgcuccagaacaaggugcagcucaaggggagggaccuccucacccugaaaaacuucaccggagaagagaucaaguacaugcuguggcugucagccgaccucaaauuccggaucaagcagaagggcgaauaccuuccuuugcugcagggaaagucccuggggaugaucuucgagaagcgcagcacucgcacuagacugucaacugaaaccggcuucgcgcugcugggaggacaccccugcuuccugaccacccaagauauccaucugggugugaacgaaucccucaccgacacagcgcgggugcugucguccauggcagacgcgguccucgcccgcguguacaagcagucugaucuggacacucuggccaaggaagccuccauuccuaucauuaauggauuguccgaccucuaccaucccauccagauucuggccgauuaucugacucugcaagaacauuacagcucccugaaggggcuuacccuuucguggaucggcgacggcaacaacauucugcacagcauuaugaugagcgcugccaaguuuggaaugcaccuccaagcagcgaccccgaagggauacgagccagacgccuccgugacgaagcuggcugagcaguacgccaaggagaacggcacuaagcugcugcucaccaacgacccucucgaagccgcccacgguggcaacgugcugaucaccgauaccuggaucuccaugggacaggaggaggaaaagaagaagcgccugcaagcauuucagggguaccaggugacuaugaaaaccgccaaggucgccgccucggacuggaccuucuugcacugucugcccagaaagcccgaagagguggacgacgagguguucuacagcccgcggucgcuggucuuuccggaggccgaaaacaggaaguggacuaucauggccgugauggugucccugcugaccgauuacuccccgcagcugcagaaaccaaaguucugacggguggcaucccugugaccccuccccagugccucuccuggcccuggaaguugccacuccagugcccaccagccuuguccuaauaaaauuaaguugcaucaagcu

SEQ ID NO: 5 - RNA, 1310 nt, Artificial Sequence
  chemically synthesized oligonucleotide
ggacagaucgccuggagacgccauccacgcuguuuugaccuccauagaagacaccgggaccgauccagccuccgcggccgggaacggugcauuggaacgcggauuccccgugccaagagugacucaccguccuugacacgaugcuguucaaccuucggaucuugcugaacaacgcugcguuccggaauggucacaacuucaugguccggaacuucagaugcggccagccgcuccagaacaaggugcagcucaaggggagggaccuccucacccugaaaaacuucaccggagaagagaucaaguacaugcuguggcugucagccgaccucaaauuccggaucaagcagaagggcgaauaccuuccuuugcugcagggaaagucccuggggaugaucuucgagaagcgcagcacucgcacuagacugucaacugaaaccggcuucgcgcugcugggaggacaccccugcuuccugaccacccaagauauccaucugggugugaacgaaucccucaccgacacagcgcgggugcugucguccauggcagacgcgguccucgcccgcguguacaagcagucugaucuggacacucuggccaaggaagccuccauuccuaucauuaauggauuguccgaccucuaccaucccauccagauucuggccgauuaucugacucugcaagaacauuacagcucccugaaggggcuuacccuuucguggaucggcgacggcaacaacauucugcacagcauuaugaugagcgcugccaaguuuggaaugcaccuccaagcagcgaccccgaagggauacgagccagacgccuccgugacgaagcuggcugagcaguacgccaaggagaacggcacuaagcugcugcucaccaacgacccucucgaagccgcccacgguggcaacgugcugaucaccgauaccuggaucuccaugggacaggaggaggaaaagaagaagcgccugcaagcauuucagggguaccaggugacuaugaaaaccgccaaggucgccgccucggacuggaccuucuugcacugucugcccagaaagcccgaagagguggacgacgagguguucuacagcccgcggucgcuggucuuuccggaggccgaaaacaggaaguggacuaucauggccgugauggugucccugcugaccgauuacuccccgcagcugcagaaaccaaaguucugaggguggcaucccugugaccccuccccagugccucuccuggcccuggaaguugccacuccagugcccaccagccuuguccuaauaaaauuaaguugcaucaaagcu

SEQ ID NO: 6 - RNA, 1310 nt, Artificial Sequence
  chemically synthesized oligonucleotide
ggacagaucgccuggagacgccauccacgcuguuuugaccuccauagaagacaccgggaccgauccagccuccgcggccgggaacggugcauuggaacgcggauuccccgugccaagagugacucaccguccuugacacgaugcuguuuaaccugagaauucugcugaacaacgccgcguucaggaacggccacaauuucaugguccgcaacuuuagaugcggacagccucuccaaaacaagguccagcucaaggggcgggacuugcugacccuuaagaacuuuaccggcgaagagaucaaguacaugcugugguugucagcggaccugaaguuccgcaucaagcagaaaggggaguaucugccgcugcuccaaggaaagucgcucggcaugaucuucgagaagcgcucgaccagaacccggcuguccacugaaacugguuucgcccuucuggguggacacccuuguuuccugacaacccaggacauccaucugggcgugaacgaaagccucacugacaccgccagggugcugagcuccauggccgacgcuguccuugcccggguguacaagcaguccgaucuggacacucuggccaaggaagcguccaucccgaucauuaacggacuguccgaccuguaccacccgauccagauucuggccgacuaccugaccuugcaagagcacuacagcucacugaagggcuugacccugagcuggaucggcgacggaaacaacauucugcauucgaucaugauguccgcggccaaguucggaaugcaucugcaggccgcaacucccaagggauacgaaccugaugcguccgugacuaagcuggccgagcaguacgcaaaggaaaacggcaccaagcugcugcugaccaacgacccgcucgaagcugcccacggagggaacgugcucauuaccgacacuuggaucuccauggggcaggaagaagagaagaagaagcggcuccaggcauuccaggguuaccaggucaccaugaaaacggccaaaguggccgcuucggauuggacuuuccuccacugccuuccccgcaaaccugaggaaguggaugaugaaguguucuacuccccacgcucccucguguuccccgaggccgagaaucggaaguggaccauuauggccgugauggugucacugcugaccgacuacagcccccaacugcaaaagccgaaguucugacggguggcaucccugugaccccuccccagugccucuccuggcccuggaaguugccacuccagugcccaccagccuuguccuaauaaaauuaaguugcaucaagcu

SEQ ID NO: 7 - RNA, 1239 nt, Artificial Sequence
  chemically synthesized oligonucleotide
augagcagcaagggcagcguggugcuggccuacagcggcggccuggacaccagcugcauccugguguggcugaaggagcagggcuacgacgugaucgccuaccuggccaacaucggccagaaggaggacuucgaggaggcccgcaagaaggcccugaagcugggcgccaagaagguguucaucgaggacgugagccgcgaguucguggaggaguucaucuggcccgccauccagagcagcgcccuguacgaggaccgcuaccugcugggcaccagccuggcccgccccugcaucgcccgcaagcagguggagaucgcccagcgcgagggcgccaaguacgugagccacggcgccaccggcaagggcaacgaccaggugcgcuucgagcugagcugcuacagccuggccccccagaucaaggugaucgcccccuggcgcaugcccgaguucuacaaccgcuucaagggccgcaacgaccugauggaguacgccaagcagcacggcauccccauccccgugacccccaagaaccccuggagcauggacgagaaccugaugcacaucagcuacgaggccggcauccuggagaaccccaagaaccaggccccccccggccuguacaccaagacccaggaccccgccaaggcccccaacacccccgacauccuggagaucgaguucaagaagggcgugcccgugaaggugaccaacgugaaggacggcaccacccaccagaccagccuggagcuguucauguaccugaacgagguggccggcaagcacggcgugggccgcaucgacaucguggagaaccgcuucaucggcaugaagagccgcggcaucuacgagacccccgccggcaccauccuguaccacgcccaccuggacaucgaggccuucaccauggaccgcgaggugcgcaagaucaagcagggccugggccugaaguucgccgagcugguguacaccggcuucuggcacagccccgagugcgaguucgugcgccacugcaucgccaagagccaggagcgcguggagggcaaggugcaggugagcgugcugaagggccagguguacauccugggccgcgagagcccccugagccuguacaacgaggagcuggugagcaugaacgugcagggcgacuacgagcccaccgacgccaccggcuucaucaacaucaacagccugcgccugaaggaguaccaccgccugcagagcaaggugaccgccaaguga

SEQ ID NO: 8 - RNA, 1359 nt, Artificial Sequence
  chemically synthesized oligonucleotide
augagcaccgccgugcuggagaaccccggccugggccgcaagcugagcgacuucggccaggagaccagcuacaucgaggacaacugcaaccagaacggcgccaucagccugaucuucagccugaaggaggaggugggcgcccuggccaaggugcugcgccuguucgaggagaacgacgugaaccugacccacaucgagagccgccccagccgccugaagaaggacgaguacgaguucuucacccaccuggacaagcgcagccugcccgcccugaccaacaucaucaagauccugcgccacgacaucggcgccaccgugcacgagcugagccgcgacaagaagaaggacaccgugcccugguucccccgcaccauccaggagcuggaccgcuucgccaaccagauccugagcuacggcgccgagcuggacgccgaccaccccggcuucaaggaccccguguaccgcgcccgccgcaagcaguucgccgacaucgccuacaacuaccgccacggccagcccaucccccgcguggaguacauggaggaggagaagaagaccuggggcaccguguucaagacccugaagagccuguacaagacccacgccugcuacgaguacaaccacaucuucccccugcuggagaaguacugcggcuuccacgaggacaacaucccccagcuggaggacgugagccaguuccugcagaccugcaccggcuuccgccugcgccccguggccggccugcugagcagccgcgacuuccugggcggccuggccuuccgcguguuccacugcacccaguacauccgccacggcagcaagcccauguacacccccgagcccgacaucugccacgagcugcugggccacgugccccuguucagcgaccgcagcuucgcccaguucagccaggagaucggccuggccagccugggcgcccccgacgaguacaucgagaagcuggccaccaucuacugguucaccguggaguucggccugugcaagcagggcgacagcaucaaggccuacggcgccggccugcugagcagcuucggcgagcugcaguacugccugagcgagaagcccaagcugcugccccuggagcuggagaagaccgccauccagaacuacaccgugaccgaguuccagccccuguacuacguggccgagagcuucaacgacgccaaggagaaggugcgcaacuucgccgccaccaucccccgccccuucagcgugcgcuacgaccccuacacccagcgcaucgaggugcuggacaacacccagcagcugaagauccuggccgacagcaucaacagcgagaucggcauccugugcagcgcccugcagaagaucaaguaa